European Patent Application EP 4 112 728 A1, published January 4, 2023. Title: METHOD FOR IDENTIFYING TARGET-BINDING PEPTIDES. Applicant: ETH Zürich. The sequence listing filed with the application follows.

SEQUENCE LISTING (22 sequences)

SEQ ID NO: 1 - protein, 25 aa, Artificial Sequence
  Meucin-25
VKLIQIRIWIQYVTVLQMFSMKTKQ

SEQ ID NO: 2 - protein, 24 aa, Artificial Sequence
  Ascaphin-6
GFKDWIKGAAKKLIKTVASSIANE

SEQ ID NO: 3 - protein, 14 aa, Artificial Sequence
  P-10
VSKIKKYLKYKDRI

SEQ ID NO: 4 - protein, 40 aa, Artificial Sequence
  Enterocin RJ-11
AIAKLVAKFGWPIVKKYYKQIMQFIGEGWAINKIIEWIKK

SEQ ID NO: 5 - protein, 31 aa, Artificial Sequence
  PepG1
MITISTMLQFGLFLIALIGLVIKLIELSIKK

SEQ ID NO: 6 - protein, 31 aa, Artificial Sequence
  PepG1
LVTLSAMLQFGIFLIAFIGLVIDLIKLSQKK

SEQ ID NO: 7 - protein, 32 aa, Artificial Sequence
  YFGAP
VKVGVNGFGRIGRLVTRAAFNSGKVEIVAIND

SEQ ID NO: 8 - protein, 30 aa, Artificial Sequence
  PepG1
MITISTMLQFGLFLIALIGLVIKLIELSNK

SEQ ID NO: 9 - protein, 32 aa, Artificial Sequence; identical to SEQ ID NO: 7
  YFGAP

SEQ ID NO: 10 - protein, 18 aa, Artificial Sequence
  Pyrrhocoricin
VDKGGYLPRPTPPRPVYR

SEQ ID NO: 11 - protein, 23 aa, Artificial Sequence
  Latarcin 4a
LKDKVKSMGEKLKQYIQTWKAKF

SEQ ID NO: 12 - protein, 30 aa, Artificial Sequence
  PepG1
LVYISIMLQFGMFIIAFIGLVIELIKLRQK

SEQ ID NO: 13 - protein, 27 aa, Artificial Sequence
  Vv-AMP1
RACESQSHRFKGTCVRQSNCAAVCQTE

SEQ ID NO: 14 - protein, 34 aa, Artificial Sequence
  BF-CATH
KRFKKFFKKLKKSVKKRAKKFFKKPRVIGVSIPF

SEQ ID NO: 15 - protein, 24 aa, Artificial Sequence
  Delta Lysine 1
MAADIISTIGDLVKWIIDTVNKFK

SEQ ID NO: 16 - protein, 16 aa, Artificial Sequence
  Maximin 3
TALKGAAKELASTYQH

SEQ ID NO: 17 - protein, 26 aa, Artificial Sequence
  PepG1
PMLQFGLFLIALIGLVIKLIELSNKK

SEQ ID NO: 18 - protein, 37 aa, Artificial Sequence
  Oxyopinin 2b
GKFSGFAKILKSIAKFFKGVGKVRKGFKEASDLDKNQ

SEQ ID NO: 19 - protein, 32 aa, Artificial Sequence
  Cycloviolacin H2
SYIPCGESCVYIPCTVTALLGCSCSNKVCYKN

SEQ ID NO: 20 - protein, 37 aa, Artificial Sequence
  HFIAP-1
GWFKKAWRKVKHAGRRVLDTAKGVGRHYLNNWLNRYR

SEQ ID NO: 21 - DNA, 18 bp, Artificial Sequence
  Primer 1
ctgcacaaagcttacgtg

SEQ ID NO: 22 - DNA, 18 bp, Artificial Sequence
  Primer 2
cacgtaagctttgtgcag